European Patent Specification EP 3 415 159 B1, published December 13, 2023. Title: Pre-treatment drug of T cell infusion therapy against tumors with the resistance to the immune checkpoint inhibitor. Applicant: MIE UNIVERSITY KYOTO UNIVERSITY. The sequence listing filed with the application follows.

SEQUENCE LISTING (3 sequences)

SEQ ID NO: 1 - protein, 38 aa, Artificial
  MEN peptide
SNPARYEFLYYYYYYQYIHSANVLYYYYYYRGPESRLL

SEQ ID NO: 2 - protein, 37 aa, Artificial
  p121 peptide
NDHIAYFLYQILRGLQYIHSANVLHRDLKPSNLLLNT

SEQ ID NO: 3 - protein, 9 aa, Artificial
  CD8+ epitope
QYIHSANVL